European Patent Specification EP 3 684 796 B1, published February 26, 2025. Title: SUCCINATE-REGULATING POLYPEPTIDES AND USE THEREOF. Applicant: B. G. NEGEV TECHNOLOGIES AND APPLICATIONS LTD., AT BEN-GURION UNIVERSITY. The sequence listing filed with the application follows.

SEQUENCE LISTING (23 sequences)

SEQ ID NO: 1 - protein, 735 aa, Mus musculus
MELQRRDYHVERPLLNQEQLEDLGHWGPAAKTHQWRTWFRCSRARAHSLLLQHVPVLGWLPRYPVREWLLGDLLSGLSVAIMQLPQGLAYALLAGLPPMFGLYSSFYPVFIYFLFGTSRHISVGTFAVMSVMVGSVTESLTADKAFVQGLNATADDARVQVAYTLSFLVGLFQVGLGLVHFGFVVTYLSEPLVRSYTTAASVQVLVSQLKYVFGIKLSSHSGPLSVIYTVLEVCAQLPETVPGTVVTAIVAGVALVLVKLLNEKLHRRLPLPIPGELLTLIGATGISYGVKLNDRFKVDVVGNITTGLIPPVAPKTELFATLVGNAFAIAVVGFAIAISLGKIFALRHGYRVDSNQELVALGLSNLIGGFFQCFPVSCSMSRSLVQESTGGNTQVAGAVSSLFILLIIVKLGELFRDLPKAVLAAVIIVNLKGMMKQFSDICSLWKANRVDLLIWLVTFVATILLNLDIGLAVSIVFSLLLVVVRMQLPHYSVLGQVPDTDIYRDVAEYSGAKEVPGVKVFRSSATLYFANAELYSDSLKEKCGVDVDRLITQKKKRIKKQEMKLKRMKKAKKSQKQDASSKISSVSVNVNTNLEDVKSNDVEGSEAKVHQGEELQDVVSSNQEDAKAPTMTSLKSLGLPQPGFHSLILDLSTLSFVDTVCIKSLKNIFRDFREIEVEVYIAACYSPVVAQLEAGHFFDESITKQHVFASVHDAVTFALSHRKSVPKSPVLATKL

SEQ ID NO: 2 - protein, 759 aa, Homo sapiens
MGLADASGPRDTQALLSATQAMDLRRRDYHMERPLLNQEHLEELGRWGSAPRTHQWRTWLQCSRARAYALLLQHLPVLVWLPRYPVRDWLLGDLLSGLSVAIMQLPQGLAYALLAGLPPVFGLYSSFYPVFIYFLFGTSRHISVGTFAVMSVMVGSVTESLAPQALNDSMINETARDAARVQVASTLSVLVGLFQVGLGLIHFGFVVTYLSEPLVRGYTTAAAVQVFVSQLKYVFGLHLSSHSGPLSLIYTVLEVCWKLPQSKVGTVVTAAVAGVVLVVVKLLNDKLQQQLPMPIPGELLTLIGATGISYGMGLKHRFEVDVVGNIPAGLVPPVAPNTQLFSKLVGSAFTIAVVGFAIAISLGKIFALRHGYRVDSNQELVALGLSNLIGGIFQCFPVSCSMSRSLVQESTGGNSQVAGAISSLFILLIIVKLGELFHDLPKAVLAAIIIVNLKGMLRQLSDMRSLWKANRADLLIWLVTFTATILLNLDLGLVVAVIFSLLLVVVRTQMPHYSVLGQVPDTDIYRDVAEYSEAKEVRGVKVFRSSATVYFANAEFYSDALKQRCGVDVDFLISQKKKLLKKQEQLKLKQLQKEEKLRKQAASPKGASVSINVNTSLEDMRSNNVEDCKMMQVSSGDKMEDATANGQEDSKAPDGSTLKALGLPQPDFHSLILDLGALSFVDTVCLKSLKNIFHDFREIEVEVYMAACHSPVVSQLEAGHFFDASITKKHLFASVHDAVTFALQHPRPVPDSPVSVTRL

SEQ ID NO: 3 - protein, 530 aa, Mus musculus
MSMPDAMPLPGVGEELKQAKEIEDAEKYSFMATVTKAPKKQIQFADDMQEFTKFPTKTGRRSLSRSISQSSTDSYSSAASYTDSSDDEVSPREKQQTNSKGSSNFCVKNIKQAEFGRREIEIAEQDMSALISLRKRAQGEKPLAGAKIVGCTHITAQTAVLIETLCALGAQCRWSACNIYSTQNEVAAALAEAGVAVFAWKGESEDDFWWCIDRCVNMDGWQANMILDDGGDLTHWVYKKYPNVFKKIRGIVEESVTGVHRLYQLSKAGKLCVPAMNVNDSVTKQKFDNLYCCRESILDGLKRTTDVMFGGKQVVVCGYGEVGKGCCAALKALGAIVYITEIDPICALQACMDGFRVVKLNEVIRQVDVVITCTGNKNVVTREHLDRMKNSCIVCNMGHSNTEIDVTSLRTPELTWERVRSQVDHVIWPDGKRVVLLAEGRLLNLSCSTVPTFVLSITATTQALALIELYNAPEGRYKQDVYLLPKKMDEYVASLHLPSFDAHLTELTDDQAKYLGLNKNGPFKPNYYRY

SEQ ID NO: 4 - protein, 530 aa, Homo sapiens; identical to SEQ ID NO: 3

SEQ ID NO: 5 - protein, 585 aa, Mus musculus
MATCWQALWAYRSYLIVLCLPIFLLPLPLIVQTKEAYCAYSIILMALLWCTEALPLAVTALFPIILFPLMGIMEASKVCLEYFKDTNILFVGGLMVAIAVEHWNLHKRIALGVLLIIGVRPALLLLGFMLVTAFLSMWISNTATTAMMLPIGYAVLEQLQGSQKDVEEGNSNPSFELQEASPQKEETKLDNGQAVSVSSEPRAQKTKEHHRFSQGLSLCICYSASIGGIATLTGTTPNLVLQGQVNSIFPENSNVVNFASWFGFAFPTMVILLLLAWLWLQVLFLGVNFRKNFGFGEGEEERKQAAFQVIKTQHRLLGPMSFAEKAVTFLFVLLVVLWFTREPGFFPGWGDTAFANKGQSMVSDGTVAIFISLIMFIIPSKIPGLTEDPKKPGKLKAPPAILTWKTVNDKMPWNILILLGGGFALAKGSEESGLSKWLGDKLTPLQHVPPSATVLILSLLVAIFTECTSNVATTTLFLPILASMAQAICLHPLYVMLPCTLAASLAFMLPVATPPNAIVFSFGGLKVSDMARAGFLLNIIGVLTITLSINSWSIPIFKLDTFPTWAYSNTSQCLLNPPNSTVPGH

SEQ ID NO: 6 - protein, 641 aa, Homo sapiens
MATCWQALWAYRSYLIVFFVPILLLPLPILVPSKEAYCAYAIILMALFWCTEALPLAVTALFPLILFPMMGIVDASEIIQRPFPSSFESPGECQSVGMSVTASHNLGGTVGDSRVFPPLSHVSTCQVAVEYLKDSNLLFFGGLLVAIAVEHWNLHKRIALRVLLIVGVRPAPLILGFMLVTAFLSMWISNTATSAMMVPIAHAVLDQLHSSQASSNVEEGSNNPTFELQEPSPQKEVTKLDNGQALPVTSASSEGRAHLSQKHLHLTQCMSLCVCYSASIGGIATLTGTAPNLVLQGQINSLFPQNGNVVNFASWFSFAFPTMVILLLLAWLWLQILFLGFNFRKNFGIGEKMQEQQQAAYCVIQTEHRLLGPMTFAEKAISILFVILVLLWFTREPGFFLGWGNLAFPNAKGESMVSDGTVAIFIGIIMFIIPSKFPGLTQDPENPGKLKAPLGLLDWKTVNQKMPWNIVLLLGGGYALAKGSERSGLSEWLGNKLTPLQSVPAPAIAIILSLLVATFTECTSNVATTTIFLPILASMAQAICLHPLYVMLPCTLATSLAFMLPVATPPNAIVFSFGDLKVLDMARAGFLLNIIGVLIIALAINSWGIPLFSLHSFPSWAQSNTTAQCLPSLANTTTPSP

SEQ ID NO: 7 - protein, 334 aa, Homo sapiens
MLGIMAWNATCKNWLAAEAALEKYYLSIFYGIEFVVGVLGNTIVVYGYIFSLKNWNSSNIYLFNLSVSDLAFLCTLPMLIRSYANGNWIYGDVLCISNRYVLHANLYTSILFLTFISIDRYLIIKYPFREHLLQKKEFAILISLAIWVLVTLELLPILPLINPVITDNGTTCNDFASSGDPNYNLIYSMCLTLLGFLIPLFVMCFFYYKIALFLKQRNRQVATALPLEKPLNLVIMAVVIFSVLFTPYHVMRNVRIASRLGSWKQYQCTQVVINSFYIVTRPLAFLNSVINPVFYFLLGDHFRDMLMNQLRHNFKSLTSFSRWAHELLLSFREK

SEQ ID NO: 8 - DNA, 1005 bp, Homo sapiens
atgctggggatcatggcatggaatgcaacttgcaaaaactggctggcagcagaggctgccctggaaaagtactacctttccattttttatgggattgagttcgttgtgggagtccttggaaataccattgttgtttacggctacatcttctctctgaagaactggaacagcagtaatatttatctctttaacctctctgtctctgacttagcttttctgtgcaccctccccatgctgataaggagttatgccaatggaaactggatatatggagacgtgctctgcataagcaaccgatatgtgcttcatgccaacctctataccagcattctctttctcacttttatcagcatagatcgatacttgataattaagtatcctttccgagaacaccttctgcaaaagaaagagtttgctattttaatctccttggccatttgggttttagtaaccttagagttactacccatacttccccttataaatcctgttataactgacaatggcaccacctgtaatgattttgcaagttctggagaccccaactacaacctcatttacagcatgtgtctaacactgttggggttccttattcctctttttgtgatgtgtttcttttattacaagattgctctcttcctaaagcagaggaataggcaggttgctactgctctgccccttgaaaagcctctcaacttggtcatcatggcagtggtaatcttctctgtgctttttacaccctatcacgtcatgcggaatgtgaggatcgcttcacgcctggggagttggaagcagtatcagtgcactcaggtcgtcatcaactccttttacattgtgacacggcctttggcctttctgaacagtgtcatcaaccctgtcttctattttcttttgggagatcacttcagggacatgctgatgaatcaactgagacacaacttcaaatcccttacatcctttagcagatgggctcatgaactcctactttcattcagagaaaagtga

SEQ ID NO: 9 - protein, 60 aa, Vibrio cholerae
  misc_feature (18)..(18): Xaa can be any naturally occurring amino acid
  misc_feature (34)..(34): Xaa can be any naturally occurring amino acid
  misc_feature (39)..(39): Xaa can be any naturally occurring amino acid
  misc_feature (45)..(45): Xaa can be any naturally occurring amino acid
  misc_feature (55)..(55): Xaa can be any naturally occurring amino acid
ANSIIFLFLGGFALAAAXHHQGLDKVIADKVLAXAQGKXSVAVFXLFGVTALLSXWISNT

SEQ ID NO: 10 - protein, 60 aa, Staphylococcus aureus
GNDIIFLFLGGFILAIAMERWNLHTRVALTIINLIGASTSKILLGFMVATGFLSMFVSNT

SEQ ID NO: 11 - protein, 60 aa, Drosophila melanogaster
FKDTLVMFMGGIMVALAVEYCNLHKRLALRVIQIVGCSPRRLHFGLIMVTMFLSMWISNA

SEQ ID NO: 12 - protein, 60 aa, Homo sapiens
LKDSNLLFFGGLLVAIAVEHWNLHKRIALRVLLIVGVRPAPLILGFMLVTAFLSMWISNT

SEQ ID NO: 13 - protein, 61 aa, Mus musculus
FKDTNILFVGGLMVAIAVEHWNLHKRIALGVILLIIGVRPALLLLGFMLVTAFLSMWISNT

SEQ ID NO: 14 - protein, 60 aa, Homo sapiens
FLDTNFLFLSGLIMASAIEEWNLHRRIALKILMLVGVQPARLILGMMVTTSFLSMWLSNT

SEQ ID NO: 15 - protein, 60 aa, Mus musculus
FLDTNFLFLSGLIMASAIEEWNLHRRIALKVLMLVGVQPARLILGMMVTTSFLSMWLSNT

SEQ ID NO: 16 - protein, 60 aa, Homo sapiens
MKDTNMLFLGGLIVAVAVERWNLHKRIALRTLLWVGAKPARLMLGFMGVTALLSMWISNT

SEQ ID NO: 17 - protein, 60 aa, Mus musculus
MKDTNMLFLGSLIVAVAVERWKLHKRVALRMLLFVGTKPSRLMLGFMFVTAFLSMWISNT

SEQ ID NO: 18 - protein, 60 aa, Homo sapiens
FKDFHLLLIGVICLATSIEKWNLHKRIALKMVMMVGVNPAWLTLGFMSSTAFLSMWLSNT

SEQ ID NO: 19 - protein, 60 aa, Mus musculus
FKDFHLLLIVGICLATSIEKWNLHKRIALRMVMMVGVNPAWLTLGFMSSTAFLSMWLSNT

SEQ ID NO: 20 - protein, 60 aa, Homo sapiens
FKNTTLLLVGVICVAAAVEKWNLHKRIALRMVLMAGAKPGMLLLCFMCCTTLLSMWLSNT

SEQ ID NO: 21 - protein, 63 aa, Homo sapiens
EEKLRKQAASPKGASVSINVNTSLEDMRSNNVEDCKMMQVSSGDKMEDATANGQEDSKAPDGS

SEQ ID NO: 22 - protein, 62 aa, Mus musculus
AKKSQKQDASSKISSVSVNVNTNLEDVKSNDVEGSEAKVHQGEELQDVVSSNQEDAKAPTMT

SEQ ID NO: 23 - protein, 57 aa, Sus scrofa
GNKLVKKDTSISINVNTGITNIESNDVEGSNVKVSAEKELEDIAAGDQEDAKAPAMS